European Patent Application EP 4 183 870 A1, published May 24, 2023. Title: METHOD OF CULTURING STEM CELLS. Applicant: SHANGHAI WOLWO STEM CELL TECHNOLOGY CO.,LTD. The sequence listing filed with the application follows.

SEQUENCE LISTING (16 sequences)

SEQ ID NO: 1 - DNA, 20 bp, Artificial Sequence
  Primer
ttcgtcatgggtgtgaacca

SEQ ID NO: 2 - DNA, 21 bp, Artificial Sequence
  Primer
ctgtggtcatgagtccttcca

SEQ ID NO: 3 - DNA, 21 bp, Artificial Sequence
  Primer
gaggttggctctgactgtacc

SEQ ID NO: 4 - DNA, 21 bp, Artificial Sequence
  Primer
tccgtcccagtagattaccac

SEQ ID NO: 5 - DNA, 22 bp, Artificial Sequence
  Primer
tcactgtcttgtacccttgtgc

SEQ ID NO: 6 - DNA, 20 bp, Artificial Sequence
  Primer
ggattagggcttcctcttgg

SEQ ID NO: 7 - DNA, 19 bp, Artificial Sequence
  Primer
atggagccttcggctgact

SEQ ID NO: 8 - DNA, 21 bp, Artificial Sequence
  Primer
gtaactattcggtgcgttggg

SEQ ID NO: 9 - DNA, 24 bp, Artificial Sequence
  Primer
gcatccgactgtaaagaatcttca

SEQ ID NO: 10 - DNA, 23 bp, Artificial Sequence
  Primer
catctcagcagaagacatttgca

SEQ ID NO: 11 - DNA, 19 bp, Artificial Sequence
  Primer
gggaatggaccttgtatag

SEQ ID NO: 12 - DNA, 20 bp, Artificial Sequence
  Primer
gcaaagctcctaccgtacca

SEQ ID NO: 13 - DNA, 18 bp, Artificial Sequence
  Primer
gccgcactgagatggaag

SEQ ID NO: 14 - DNA, 18 bp, Artificial Sequence
  Primer
aatgtcgagggtcccaca

SEQ ID NO: 15 - DNA, 19 bp, Artificial Sequence
  Primer
gggagaagacactgcgtca

SEQ ID NO: 16 - DNA, 18 bp, Artificial Sequence
  Primer
ggaagcactgggggaagt